European Patent Specification EP 3 589 652 B1, published December 25, 2024. Title: RECOMBINANT ANTIBODY TO PROGRAMMED DEATH 1 (PD-1) AND USES THEREOF. Applicant: Shenzhen RunShin Bioscience ZHANG, YING. The sequence listing filed with the application follows.

SEQUENCE LISTING (80 sequences)

SEQ ID NO: 1 - protein, 8 aa, Rabbit
GFTLSSYA

SEQ ID NO: 2 - protein, 8 aa, Rabbit
SNAGNGNT

SEQ ID NO: 3 - protein, 6 aa, Rabbit
YWYFDL

SEQ ID NO: 4 - protein, 8 aa, Rabbit
GFSISSYG

SEQ ID NO: 5 - protein, 8 aa, Rabbit
ISYDGSNK

SEQ ID NO: 6 - protein, 9 aa, Rabbit
YYYYYGMDV

SEQ ID NO: 7 - protein, 8 aa, Rabbit
GFTLSSYA

SEQ ID NO: 8 - protein, 8 aa, Rabbit
ISYDGSNK

SEQ ID NO: 9 - protein, 9 aa, Rabbit
YYYYYYMDV

SEQ ID NO: 10 - protein, 8 aa, Rabbit
GISLSSYY

SEQ ID NO: 11 - protein, 8 aa, Rabbit
IYYSGSTN

SEQ ID NO: 12 - protein, 5 aa, Rabbit
WYFDL

SEQ ID NO: 13 - protein, 6 aa, Rabbit
QSGSSF

SEQ ID NO: 14 - protein, 6 aa, Rabbit
ANNKRE

SEQ ID NO: 15 - protein, 9 aa, Rabbit
GTYTDSPPT

SEQ ID NO: 16 - protein, 6 aa, Rabbit
QSLSSY

SEQ ID NO: 17 - protein, 6 aa, Rabbit
DVSNRA

SEQ ID NO: 18 - protein, 9 aa, Rabbit
QQRTNWPRA

SEQ ID NO: 19 - protein, 6 aa, Rabbit
QSVSSY

SEQ ID NO: 20 - protein, 6 aa, Rabbit
EASNRA

SEQ ID NO: 21 - protein, 9 aa, Rabbit
QQRTNWPPA

SEQ ID NO: 22 - protein, 6 aa, Rabbit
NSVSSS

SEQ ID NO: 23 - protein, 6 aa, Rabbit
DTSNRE

SEQ ID NO: 24 - protein, 9 aa, Rabbit
QQRDNWPRA

SEQ ID NO: 25 - protein, 8 aa, human
GYTFTSYA

SEQ ID NO: 26 - protein, 8 aa, human
SNAGNGNT

SEQ ID NO: 27 - protein, 6 aa, human
YWYFDL

SEQ ID NO: 28 - protein, 8 aa, human
GFTFSSYG

SEQ ID NO: 29 - protein, 8 aa, human
ISYDGSNK

SEQ ID NO: 30 - protein, 9 aa, human
YYYYYGMDV

SEQ ID NO: 31 - protein, 8 aa, human
AFTFSSYA

SEQ ID NO: 32 - protein, 8 aa, human
ISYDGSNK

SEQ ID NO: 33 - protein, 9 aa, human
YYYYYYMDV

SEQ ID NO: 34 - protein, 8 aa, human
GGSISSYY

SEQ ID NO: 35 - protein, 8 aa, human
IYYSGSTN

SEQ ID NO: 36 - protein, 5 aa, human
WYFDL

SEQ ID NO: 37 - protein, 6 aa, human
QSGSSF

SEQ ID NO: 38 - protein, 6 aa, human
ANNKRE

SEQ ID NO: 39 - protein, 9 aa, human
GTYTDSPPT

SEQ ID NO: 40 - protein, 6 aa, human
QSLSSY

SEQ ID NO: 41 - protein, 6 aa, human
DVSNRA

SEQ ID NO: 42 - protein, 9 aa, human
QQRTNWPRA

SEQ ID NO: 43 - protein, 6 aa, human
QSVSSY

SEQ ID NO: 44 - protein, 6 aa, human
EASNRA

SEQ ID NO: 45 - protein, 9 aa, human
QQRTNWPPA

SEQ ID NO: 46 - protein, 6 aa, human
NSVSSS

SEQ ID NO: 47 - protein, 6 aa, human
DTSNRE

SEQ ID NO: 48 - protein, 9 aa, human
QQRDNWPRA

SEQ ID NO: 49 - DNA, 345 bp, Rabbit
tgccagagcgtggaagaaagcgaaggcggcctggtgaaaccgggcgcgagcctgaccctgagctgcaccgcgagcggctttaccctgagcagctatgcgatgcattgggtgcgccaggcgccgggcaacggcctggaatggattggctggagcaacgcgggcaacggcaacaccaaatatagccaggaatttcagggccgctttaccattacccgcaacaccagcctgagcaccgtgaccctggaaatgaccagcctgaccgcggcggataccgcgacctatttttgcgcgcgctattggtattttgatctgtggggcccgggcaccctggtgaccgtgagcagc

SEQ ID NO: 50 - protein, 115 aa, Rabbit
CQSVEESEGGLVKPGASLTLSCTASGFTLSSYAMHWVRQAPGNGLEWIGWSNAGNGNTKYSQEFQGRFTITRNTSLSTVTLEMTSLTAADTATYFCARYWYFDLWGPGTLVTVSS

SEQ ID NO: 51 - DNA, 330 bp, Rabbit
gaactggtgctgacccagaccccgagcagcgtgagcgcggcggtgggcggcaccgtgaccattaactgccaggcgagccagagcggcagcagctttgtggcgtggtatcagcagaaaccgggccagccgccgaaactgctgatttatgcgaacaacaaacgcgaaaccggcgtgccgagccgctttagcggcagcggcagcggcaccgattttaccctgaccattagcagcctggaatgcgaagatgcggcgacctattattgcggcacctataccgatagcccgccgacctttggcggcggcaccaaagtggtggtgaaaggcgatccg

SEQ ID NO: 52 - protein, 110 aa, Rabbit
ELVLTQTPSSVSAAVGGTVTINCQASQSGSSFVAWYQQKPGQPPKLLIYANNKRETGVPSRFSGSGSGTDFTLTISSLECEDAATYYCGTYTDSPPTFGGGTKVVVKGDP

SEQ ID NO: 53 - DNA, 354 bp, Rabbit
caggaaagcgtgaaagaaagcggcggcggcctggtgaaaccgggcgataccctgaccctgacctgcaaagtgagcggctttagcattagcagctatggcatgcattgggtgcgccaggcgccgggcaaaggcctggaatggattggcgtgattagctatgatggcagcaacaaatattatgcggatagcgtgaaaggccgctttaccattagccgcaacaccaaccagaacaccgtgaccctgaaaatgaccagcctgaccgcggatgataccgcgacctatttttgcgcgcgctattattattattatggcatggatgtgtggggccagggcaccctggtgaccgtgagcagc

SEQ ID NO: 54 - protein, 118 aa, Rabbit
QESVKESGGGLVKPGDTLTLTCKVSGFSISSYGMHWVRQAPGKGLEWIGVISYDGSNKYYADSVKGRFTISRNTNQNTVTLKMTSLTADDTATYFCARYYYYYGMDVWGQGTLVTVSS

SEQ ID NO: 55 - DNA, 330 bp, Rabbit
gaaattgtgctgacccagaccccgagcagcgtgagcgcggcggtgggcagcaccgtgaccattaactgccgcggcagccagagcctgagcagctatctggcgtggtatcagcagaaaccgggccagcgcccgaaactgctgatttatgatgtgagcaaccgcgcgaccggcgtgccgcgccgctttaaaggcagcggcagcggcacccagtttaccctgaccattagcggcgtgcaggcggatgatgcggcgacctattattgccagcagcgcaccaactggccgcgcgcgtttggcggcggcaccaaagtggatgtgaaaggcgatccg

SEQ ID NO: 56 - protein, 110 aa, Rabbit
EIVLTQTPSSVSAAVGSTVTINCRGSQSLSSYLAWYQQKPGQRPKLLIYDVSNRATGVPRRFKGSGSGTQFTLTISGVQADDAATYYCQQRTNWPRAFGGGTKVDVKGDP

SEQ ID NO: 57 - DNA, 345 bp, Rabbit
tgccagagcctggaagaaagcggcggcggcctggtgcagccgggcaccaccctgaccctgagctgcaccgtgagcggctttaccctgagcagctatgcgatgatgtgggtgcgccaggcgccgggcaaaggcctggaatggattggcgtgattagctatgatggcagcaacaaatattatgcgcagagcgtgaaaggccgctttaccattagccgcaacaccagccagaacaccgtgaccctgaaaatgaccagcctgaccgcggaagataccgcgacctatttttgcgcgcgctattattattattattatatggatgtgtggggcccggtgaccgtgagcagc

SEQ ID NO: 58 - protein, 115 aa, Rabbit
CQSLEESGGGLVQPGTTLTLSCTVSGFTLSSYAMMWVRQAPGKGLEWIGVISYDGSNKYYAQSVKGRFTISRNTSQNTVTLKMTSLTAEDTATYFCARYYYYYYMDVWGPVTVSS

SEQ ID NO: 59 - DNA, 333 bp, Rabbit
gaactggtgctgacccagaccccgagcagcgtgagcgcggcggtgggcggcaccgtgaccacaattacctgccgcgcgagccagagcgtgagcagctatctggcgtggtatcagcagaaaccgggccaggcgccgaaactgctgatttatgaagcgagcaaccgcgcgaccggcgtgccgagccgctttagcggcagcggcagcggcaccgaatttaccctgaccattagcggcgtgcagtgcgatgatgcagcgacctattattgccagcagcgcaccaactggccgccggcgtttggcggcggcaccaaagtggtggtgaaaggcgatccg

SEQ ID NO: 60 - protein, 110 aa, Rabbit
ELVLTQTPSSVSAAVGGTVTITCRASQSVSSYLAWYQQKPGQAPKLLIYEASNRATGVPSRFSGSGSGTEFTLTISGVQCDDAATYYCQQRTNWPPAFGGGTKVVVKGDP

SEQ ID NO: 61 - DNA, 342 bp, Rabbit
tgccagagcgtggaagaaagcggcggcggcctggtgaaaccgaccgataccctgaccctgacctgcaccgtgagcggcattagcctgagcagctattattggagctgggtgcgccaggcgccgggcaaaggcctggaatggattggctatatttattatagcggaggcagcaccaactataacccgagcctgaaaagccgcagcaccattagccgcaacaccaacaccaacaccgtgaccctgaaaatgaccagcctgaccgcggcggataccgcgacctattattgcgcgcgctggtattttgatctgtggggccagggcaccctggtgaccgtgagcagc

SEQ ID NO: 62 - protein, 114 aa, Rabbit
CQSVEESGGGLVKPTDTLTLTCTVSGISLSSYYWSWVRQAPGKGLEWIGYIYYSGSGTNYNPSLKSRSTISRNTNTNTVTLKMTSLTAADTATYYCARWYFDLWGQGTLVTVSS

SEQ ID NO: 63 - DNA, 330 bp, Rabbit
gaaattgtgctgacccagagcccgagcagcgtgagcgtgagcgtgggcagcaccgtgaccattaactgccgcgcgagcaacagcgtgagcagcagcctggcgtggtatcagcagaaaccgggccaggcgccgcgcctgctgatttatgataccagcaaccgcgaaaccggcgtgccgagccgctttagcggcagccgcagcggcaccgaatttaccctgaccattagcggcgtgcagtgcgcggatgcggcgacctattattgccagcagcgcgataactggccgcgcgcgtttggcggcggcaccaaagtggtggtgaaacgcgatgtg

SEQ ID NO: 64 - protein, 110 aa, Rabbit
EIVLTQSPSSVSVSVGSTVTINCRASNSVSSSLAWYQQKPGQAPRLLIYDTSNRETGVPSRFSGSRSGTEFTLTISGVQCADAATYYCQQRDNWPRAFGGGTKVVVKRDV

SEQ ID NO: 65 - DNA, 345 bp, human
caggtgcagctggtgcagagcggcgcggaagtgaaaaaaccgggcgcgagcgtgaaagtgagctgcaaagcgagcggctatacctttaccagctatgcgatgcattgggtgcgccaggcgccgggccagcgcctggaatggatgggctggagcaacgcgggcaacggcaacaccaaatatagccaggaatttcagggccgcgtgaccattacccgcgataccagcgcgagcaccgcgtatatggaactgagcagcctgcgcagcgaagatatggcggtgtattattgcgcgcgctattggtattttgatctgtggggccgcggcaccctggtgaccgtgagcagc

SEQ ID NO: 66 - protein, 115 aa, human
QVQLVQSGAEVKKPGASVKVSCKASGYTFTSYAMHWVRQAPGQRLEWMGWSNAGNGNTKYSQEFQGRVTITRDTSASTAYMELSSLRSEDMAVYYCARYWYFDLWGRGTLVTVSS

SEQ ID NO: 67 - DNA, 330 bp, human
gagatcgccctgacccagagccccgctacactgagtctgagccctggcgagcgcgcaacactgagttgccgggccagccagagcggctctagcttcgtggcctggtatcagcagaaaccaggccaagccccccggctcctgatctatgccaacaacaagagagagactggcatccctgcccggttctccggatcaggttccgggaccgactttacccttactatctcctctctggaaccagaagactttgctgtgtactactgcggcacctacacagattcaccccccacgttcggacaggggaccaaggtggagattaagaggaccgtg

SEQ ID NO: 68 - protein, 110 aa, human
EIALTQSPATLSLSPGERATLSCRASQSGSSFVAWYQQKPGQAPRLLIYANNKRETGIPARFSGSGSGTDFTLTISSLEPEDFAVYYCGTYTDSPPTFGQGTKVEIKRTV

SEQ ID NO: 69 - DNA, 354 bp, human
caggtgcagctggtggaaagcggcggcggcgtggtgcagccgggccgcagcctgcgcctgagctgcgcggcgagcggctttacctttagcagctatggcatgcattgggtgcgccaggcgccgggcaaaggcctggaatgggtggcggtgattagctatgatggcagcaacaaatattatgcggatagcgtgaaaggccgctttaccattagccgcgataacagcaaaaacaccctgtatctgcagatgaacagcctgcgcgcggaagataccgcggtgtattattgcgcgcgctattattattattatggcatggatgtgtggggccagggcaccaccgtgaccgtgagcagc

SEQ ID NO: 70 - protein, 118 aa, human
QVQLVESGGGVVQPGRSLRLSCAASGFTFSSYGMHWVRQAPGKGLEWVAVISYDGSNKYYADSVKGRFTISRDNSKNTLYLQMNSLRAEDTAVYYCARYYYYYGMDVWGQGTTVTVSS

SEQ ID NO: 71 - DNA, 330 bp, human
gagattgtcctgactcagtctcccgctaccctttccttgtctccaggcgaacgggccaccattagctgccgcggaagccagagcctgtcctcatacctcgcttggtatcaacagcggcctggacaggcacccaggctgctgatctacgacgtgagcaaccgggccacagggatccccgcccggtttagtgggagcggtagcggcacagatttcactctgaccatcagcggcctggaacccgaggacttcgccgtgtactattgccagcagcggaccaactggcccagagccttcggccaaggcacgaaggtggagatcaagcggaccgtg

SEQ ID NO: 72 - protein, 110 aa, human
EIVLTQSPATLSLSPGERATISCRGSQSLSSYLAWYQQRPGQAPRLLIYDVSNRATGIPARFSGSGSGTDFTLTISGLEPEDFAVYYCQQRTNWPRAFGQGTKVEIKRTV

SEQ ID NO: 73 - DNA, 354 bp, human
caggtgcagctggtggatagcggcggcggcgtggtgcagccgggccgcagcctgcgcctgagctgcgcggcgagcgcgtttacctttagcagctatgcgatgcattgggtgcgccaggcgccgggcaaaggcctggaatgggtggcggtgattagctatgatggcagcaacaaatattatgcggatagcgtgaaaggccgctttaccattagccgcgataacagcaaaaacaccctgtatctgcagatgaacagcctgcgcgcggaagataccgcggtgtattattgcgcgcgctattattattattattatatggatgtgtggggcaaaggcaccaccgtgaccgtgagcagc

SEQ ID NO: 74 - protein, 118 aa, human
QVQLVDSGGGVVQPGRSLRLSCAASAFTFSSYAMHWVRQAPGKGLEWVAVISYDGSNKYYADSVKGRFTISRDNSKNTLYLQMNSLRAEDTAVYYCARYYYYYYMDVWGKGTTVTVSS

SEQ ID NO: 75 - DNA, 330 bp, human
gagatcgtgctgacgcaatcacccgccaccctgagcctgtcccctggcgagcgggctacactgagctgccgggccagtcagtcagtgagcagttacttggcttggtaccagcagaaacccggccaagccccacggctgcttatttatgaggcatccaacagagcgaccggcatccctgcccgcttctctggctctggatccgggaccgacttcactctcactatcagcagcctggaacccgaggacttcgcagtctattactgccagcagaggaccaactggcccccagcctttggtcagggcacaaaggtggaaatcaagcggaccgtg

SEQ ID NO: 76 - protein, 110 aa, human
EIVLTQSPATLSLSPGERATLSCRASQSVSSYLAWYQQKPGQAPRLLIYEASNRATGIPARFSGSGSGTDFTLTISSLEPEDFAVYYCQQRTNWPPAFGQGTKVEIKRTV

SEQ ID NO: 77 - DNA, 339 bp, human
caggtgcagctgcaggaaagcggcccgggcctggtgaaaccgagcgaaaccctgagcctgacctgcaccgtgagcggcggcagcattagcagctattattggagctggattcgccagccgccgggcaaaggcctggaatggattggctatatttattatagcggcagcaccaactataacccgagcctgaaaagccgcgtgaccattagcgtggataccagcaaaaaccagtttagcctgaaactgagcagcgtgaccgcggcggataccgcggtgtattattgcgcgtattggtattttgatctgtggggccgcggcaccctggtgaccgtgagcagc

SEQ ID NO: 78 - protein, 114 aa, human
QVQLQESGPGLVKPSETLSLTCTVSGGSISSYYWSWIRQPPGKGLEWIGYIYYSGGSTNYNPSLKSRVTISVDTSKNQFSLKLSSVTAADTAVYYCAYWYFDLWGRGTLVTVSS

SEQ ID NO: 79 - DNA, 330 bp, human
gagattgtgctgactcagtccccatccaccctgagtctgtcacccggacagaaagccactctgtcttgcagagccagcaatagcgtcagctcaagcctggcctggtatcagcagaagcccgggaaagctccccggcttatgatctacgacaccagtaaccgggaaaccggcatccctgagcgcttcagcggctctaagtctggcacagatttcagcctcacaatcagctccctggagcccggtgactttgccgtgtactactgccagcagcgggacaactggccccgggcattcggccaaggcacgaaggtgaccatcaagaggaccgtg

SEQ ID NO: 80 - protein, 110 aa, human
EIVLTQSPSTLSLSPGQKATLSCRASNSVSSSLAWYQQKPGKAPRLMIYDTSNRETGIPERFSGSKSGTDFSLTISSLEPGDFAVYYCQQRDNWPRAFGQGTKVTIKRTV